European Patent Application EP 4 242 229 A1, published September 13, 2023. Title: Antibody against human thymic stromal lymphopoietin, preparation method therefor and application thereof. Applicant: SHANGHAI MABGEEK BIOTECH. CO., LTD. The sequence listing filed with the application follows.

SEQUENCE LISTING (49 sequences)

SEQ ID NO: 1 - protein, 5 aa, Mus musculus
NSGVS

SEQ ID NO: 2 - protein, 16 aa, Mus musculus
VIWGDGSTNYHSALIS

SEQ ID NO: 3 - protein, 10 aa, Mus musculus
PDGYSGIFAY

SEQ ID NO: 4 - protein, 5 aa, Mus musculus
KYWIQ

SEQ ID NO: 5 - protein, 17 aa, Mus musculus
EIFPGTGTTYYNEIFKA

SEQ ID NO: 6 - protein, 12 aa, Mus musculus
RGDYDVYYALDY

SEQ ID NO: 7 - protein, 5 aa, Mus musculus
YSGVN

SEQ ID NO: 8 - protein, 16 aa, Mus musculus
VIWGDGSTNFHSALIS

SEQ ID NO: 9 - protein, 10 aa, Mus musculus
PDGYSGIFAY

SEQ ID NO: 10 - protein, 5 aa, Mus musculus
SFGMH

SEQ ID NO: 11 - protein, 17 aa, Mus musculus
YISSGSSNIYYADTVKG

SEQ ID NO: 12 - protein, 13 aa, Mus musculus
DGGSRRHYYVMDY

SEQ ID NO: 13 - protein, 12 aa, Mus musculus
SASSSISSNYLH

SEQ ID NO: 14 - protein, 7 aa, Mus musculus
RTSNLAS

SEQ ID NO: 15 - protein, 9 aa, Mus musculus
QLGSGILFT

SEQ ID NO: 16 - protein, 10 aa, Mus musculus
SANSGVNYIH

SEQ ID NO: 17 - protein, 7 aa, Mus musculus
TTSNLAS

SEQ ID NO: 18 - protein, 9 aa, Mus musculus
QQRSSYPFT

SEQ ID NO: 19 - protein, 12 aa, Mus musculus
SASSSLSSNYLH

SEQ ID NO: 20 - protein, 7 aa, Mus musculus
RTSNLAS

SEQ ID NO: 21 - protein, 9 aa, Mus musculus
QQGSGILVT

SEQ ID NO: 22 - protein, 11 aa, Mus musculus
KASQDVSPAVA

SEQ ID NO: 23 - protein, 7 aa, Mus musculus
SASYRYT

SEQ ID NO: 24 - protein, 9 aa, Mus musculus
QQHYSSPFT

SEQ ID NO: 25 - DNA, 354 bp, Synthetic
caggtgcagctgcaggagtctggccctggcctggtgaagccttctcagaccctgtctctgacctgtaccgtgtctggcttctctctgaccaactctggcgtgtcttgggtgagacagcctcctggcaagggcctggagtggctgggcgtgatctggggcgatggctctaccaactaccactctgccctgatctctagactgaccatctctaaggataactctaagtctaccgtgtacctgcagatgaactctctgagagccgaggataccgccgtgtactactgtgccaagcctgatggctactctggcatcttcgcctactggggccagggcaccctggtgaccgtgtcttct

SEQ ID NO: 26 - protein, 118 aa, Synthetic
QVQLQESGPGLVKPSQTLSLTCTVSGFSLTNSGVSWVRQPPGKGLEWLGVIWGDGSTNYHSALISRLTISKDNSKSTVYLQMNSLRAEDTAVYYCAKPDGYSGIFAYWGQGTLVTVSS

SEQ ID NO: 27 - protein, 448 aa, Synthetic
QVQLQESGPGLVKPSQTLSLTCTVSGFSLTNSGVSWVRQPPGKGLEWLGVIWGDGSTNYHSALISRLTISKDNSKSTVYLQMNSLRAEDTAVYYCAKPDGYSGIFAYWGQGTLVTVSSASTKGPSVFPLAPSSKSTSGGTAALGCLVKDYFPEPVTVSWNSGALTSGVHTFPAVLQSSGLYSLSSVVTVPSSSLGTQTYICNVNHKPSNTKVDKKVEPKSCDKTHTCPPCPAPELLGGPSVFLFPPKPKDTLMISRTPEVTCVVVDVSHEDPEVKFNWYVDGVEVHNAKTKPREEQYNSTYRVVSVLTVLHQDWLNGKEYKCKVSNKALPAPIEKTISKAKGQPREPQVYTLPPSRDELTKNQVSLTCLVKGFYPSDIAVEWESNGQPENNYKTTPPVLDSDGSFFLYSKLTVDKSRWQQGNVFSCSVMHEALHNHYTQKSLSLSPGK

SEQ ID NO: 28 - DNA, 324 bp, Synthetic
gagatcgtgctgacccagtctcctggcaccctgtctctgtctcctggcgagagagccaccctgagctgttctgcctcttcttctatctcttctaactacctgcactggtaccagcagaagcctggccagtctcctagactgctgatctacagaacctctaacctggcctctggcgtgcctgatagattctctggctctggctctggcaccgatttcaccctgaccatctctagactggagcctgaggatttcgccgtgtactactgtcagctgggctctggcatcctgttcaccttcggccagggcaccaagctggagatcaag

SEQ ID NO: 29 - protein, 108 aa, Synthetic
EIVLTQSPGTLSLSPGERATLSCSASSSISSNYLHWYQQKPGQSPRLLIYRTSNLASGVPDRFSGSGSGTDFTLTISRLEPEDFAVYYCQLGSGILFTFGQGTKLEIK

SEQ ID NO: 30 - protein, 215 aa, Synthetic
EIVLTQSPGTLSLSPGERATLSCSASSSISSNYLHWYQQKPGQSPRLLIYRTSNLASGVPDRFSGSGSGTDFTLTISRLEPEDFAVYYCQLGSGILFTFGQGTKLEIKRTVAAPSVFIFPPSDEQLKSGTASVVCLLNNFYPREAKVQWKVDNALQSGNSQESVTEQDSKDSTYSLSSTLTLSKADYEKHKVYACEVTHQGLSSPVTKSFNRGEC

SEQ ID NO: 31 - DNA, 363 bp, Synthetic
caggtgcagctggtgcagtctggcgccgaggtgaagaagcctggcgcctctgtgaaggtgtcttgtaagacctctggctacaccttcaccaagtactggatccagtgggtgagacaggcccctggccagggcctggagtggatcggcgagatcttccctggcaccggcaccacctactacaacgagatcttcaaggccagagtgaccctgaccgtggatacctctacctctaccgcctacatggagctgtctagcctgagatctgaggataccgccgtgtactactgtgccagaagaggcgattacgatgtgtactacgccctggattactggggccagggcaccctggtgaccgtgtcttct

SEQ ID NO: 32 - protein, 121 aa, Synthetic
QVQLVQSGAEVKKPGASVKVSCKTSGYTFTKYWIQWVRQAPGQGLEWIGEIFPGTGTTYYNEIFKARVTLTVDTSTSTAYMELSSLRSEDTAVYYCARRGDYDVYYALDYWGQGTLVTVSS

SEQ ID NO: 33 - protein, 451 aa, Synthetic
QVQLVQSGAEVKKPGASVKVSCKTSGYTFTKYWIQWVRQAPGQGLEWIGEIFPGTGTTYYNEIFKARVTLTVDTSTSTAYMELSSLRSEDTAVYYCARRGDYDVYYALDYWGQGTLVTVSSASTKGPSVFPLAPSSKSTSGGTAALGCLVKDYFPEPVTVSWNSGALTSGVHTFPAVLQSSGLYSLSSVVTVPSSSLGTQTYICNVNHKPSNTKVDKKVEPKSCDKTHTCPPCPAPELLGGPSVFLFPPKPKDTLMISRTPEVTCVVVDVSHEDPEVKFNWYVDGVEVHNAKTKPREEQYNSTYRVVSVLTVLHQDWLNGKEYKCKVSNKALPAPIEKTISKAKGQPREPQVYTLPPSRDELTKNQVSLTCLVKGFYPSDIAVEWESNGQPENNYKTTPPVLDSDGSFFLYSKLTVDKSRWQQGNVFSCSVMHEALHNHYTQKSLSLSPGK

SEQ ID NO: 34 - DNA, 318 bp, Synthetic
gagatcgtgctgacccagtctcctgccaccctgtctctgtctcctggcgagagagccaccctgtcttgttctgccaactctggcgtgaactacatccactggtaccagcagaagcctggccaggcccctagattctggatctggaccacctctaacctggcctctggcgtgcctgccagattctctggctctggctctggcaccgatttcaccctgaccatctctagcctggagcctgaggatttcgccgtgtactactgtcagcagagatcttcttaccctttcaccttcggccagggcaccaagctggagatcaag

SEQ ID NO: 35 - protein, 106 aa, Synthetic
EIVLTQSPATLSLSPGERATLSCSANSGVNYIHWYQQKPGQAPRFWIWTTSNLASGVPARFSGSGSGTDFTLTISSLEPEDFAVYYCQQRSSYPFTFGQGTKLEIK

SEQ ID NO: 36 - protein, 213 aa, Synthetic
EIVLTQSPATLSLSPGERATLSCSANSGVNYIHWYQQKPGQAPRFWIWTTSNLASGVPARFSGSGSGTDFTLTISSLEPEDFAVYYCQQRSSYPFTFGQGTKLEIKRTVAAPSVFIFPPSDEQLKSGTASVVCLLNNFYPREAKVQWKVDNALQSGNSQESVTEQDSKDSTYSLSSTLTLSKADYEKHKVYACEVTHQGLSSPVTKSFNRGEC

SEQ ID NO: 37 - DNA, 354 bp, Synthetic
gaggtgcagctggtggagtccggcggcggactggtgcagcctggaggaagcctgcggctgagctgctccgtgagcggctttagcctgacctacagcggcgtgaattgggtgaggcaggctcccggcaagggcctggagtggctgggagcaatctggggcgatggcagcaccaactaccactccgccctgatcagccggctgaccatctccaaggacaacagcaagtccaccgtgtacctgcagatgaacagcctgagggccgaggacaccgccgtgtattattgcgctaagcccgatggctattccggcatctttgcctactggggccagggcaccctggtgaccgtgtcctcc

SEQ ID NO: 38 - protein, 118 aa, Synthetic
EVQLVESGGGLVQPGGSLRLSCSVSGFSLTYSGVNWVRQAPGKGLEWLGAIWGDGSTNYHSALISRLTISKDNSKSTVYLQMNSLRAEDTAVYYCAKPDGYSGIFAYWGQGTLVTVSS

SEQ ID NO: 39 - protein, 448 aa, Synthetic
EVQLVESGGGLVQPGGSLRLSCSVSGFSLTYSGVNWVRQAPGKGLEWLGAIWGDGSTNYHSALISRLTISKDNSKSTVYLQMNSLRAEDTAVYYCAKPDGYSGIFAYWGQGTLVTVSSASTKGPSVFPLAPSSKSTSGGTAALGCLVKDYFPEPVTVSWNSGALTSGVHTFPAVLQSSGLYSLSSVVTVPSSSLGTQTYICNVNHKPSNTKVDKKVEPKSCDKTHTCPPCPAPELLGGPSVFLFPPKPKDTLMISRTPEVTCVVVDVSHEDPEVKFNWYVDGVEVHNAKTKPREEQYNSTYRVVSVLTVLHQDWLNGKEYKCKVSNKALPAPIEKTISKAKGQPREPQVYTLPPSRDELTKNQVSLTCLVKGFYPSDIAVEWESNGQPENNYKTTPPVLDSDGSFFLYSKLTVDKSRWQQGNVFSCSVMHEALHNHYTQKSLSLSPGK

SEQ ID NO: 40 - DNA, 324 bp, Synthetic
gagatcgtgctgacccagtcccctggcaccctgagcctgagccccggagagagagctaccctgagctgcagcgcaagcagctccctgagctccaattacctgcactggtatcagcagaagcctggccaggctcccaggctgctgatctacaggaccagcaacctggccagcggcgtgcctgaccggttttccggctccggctccggaaccgatttcaccctgaccatctccaggctggagcccgaggactttgccgtgtactattgtcagcagggctccggcatcctggtgaccttcggccagggcaccaagctggagatcaag

SEQ ID NO: 41 - protein, 108 aa, Synthetic
EIVLTQSPGTLSLSPGERATLSCSASSSLSSNYLHWYQQKPGQAPRLLIYRTSNLASGVPDRFSGSGSGTDFTLTISRLEPEDFAVYYCQQGSGILVTFGQGTKLEIK

SEQ ID NO: 42 - protein, 215 aa, Synthetic
EIVLTQSPGTLSLSPGERATLSCSASSSLSSNYLHWYQQKPGQAPRLLIYRTSNLASGVPDRFSGSGSGTDFTLTISRLEPEDFAVYYCQQGSGILVTFGQGTKLEIKRTVAAPSVFIFPPSDEQLKSGTASVVCLLNNFYPREAKVQWKVDNALQSGNSQESVTEQDSKDSTYSLSSTLTLSKADYEKHKVYACEVTHQGLSSPVTKSFNRGEC

SEQ ID NO: 43 - DNA, 366 bp, Synthetic
gaagtgcagctggtggagtctggcggcggcctggtgcagcctggcggctctctgagactgtcttgtgccgcctctggcttcaccttctcttctttcggcatgcactgggtgagacaggcccctggcaagggcctggagtgggtgtcctacatctcttctggctcttctaacatctactacgccgataccgtgaagggcagattcaccatctctagagataacgccaagaactctctgtacctgcagatgaactctctgagagccgaggataccgccgtgtactactgtgccagagatggcggctctagaagacactactacgtgatggattactggggccagggcaccctggtgaccgtgtcttct

SEQ ID NO: 44 - protein, 122 aa, Synthetic
EVQLVESGGGLVQPGGSLRLSCAASGFTFSSFGMHWVRQAPGKGLEWVSYISSGSSNIYYADTVKGRFTISRDNAKNSLYLQMNSLRAEDTAVYYCARDGGSRRHYYVMDYWGQGTLVTVSS

SEQ ID NO: 45 - protein, 452 aa, Synthetic
EVQLVESGGGLVQPGGSLRLSCAASGFTFSSFGMHWVRQAPGKGLEWVSYISSGSSNIYYADTVKGRFTISRDNAKNSLYLQMNSLRAEDTAVYYCARDGGSRRHYYVMDYWGQGTLVTVSSASTKGPSVFPLAPSSKSTSGGTAALGCLVKDYFPEPVTVSWNSGALTSGVHTFPAVLQSSGLYSLSSVVTVPSSSLGTQTYICNVNHKPSNTKVDKKVEPKSCDKTHTCPPCPAPELLGGPSVFLFPPKPKDTLMISRTPEVTCVVVDVSHEDPEVKFNWYVDGVEVHNAKTKPREEQYNSTYRVVSVLTVLHQDWLNGKEYKCKVSNKALPAPIEKTISKAKGQPREPQVYTLPPSRDELTKNQVSLTCLVKGFYPSDIAVEWESNGQPENNYKTTPPVLDSDGSFFLYSKLTVDKSRWQQGNVFSCSVMHEALHNHYTQKSLSLSPGK

SEQ ID NO: 46 - DNA, 321 bp, Synthetic
gagatcgtgctgacccagtctcctgccaccctgagcctgtctcctggcgagagagccaccctgtcttgtaaggcctctcaggatgtgtctcctgccgtggcctggtaccagcagaagcctggccagtcccctagactgctgatctactctgcctcttacagatacaccggcgtgcctgccagattctctggcagcggctctggcaccgatttcaccctgaccatctctagcctggagcctgaggatttcgccgtgtactactgtcagcagcactacagctctcctttcaccttcggccagggcaccaagctggagatcaag

SEQ ID NO: 47 - protein, 107 aa, Synthetic
EIVLTQSPATLSLSPGERATLSCKASQDVSPAVAWYQQKPGQSPRLLIYSASYRYTGVPARFSGSGSGTDFTLTISSLEPEDFAVYYCQQHYSSPFTFGQGTKLEIK

SEQ ID NO: 48 - protein, 214 aa, Synthetic
EIVLTQSPATLSLSPGERATLSCKASQDVSPAVAWYQQKPGQSPRLLIYSASYRYTGVPARFSGSGSGTDFTLTISSLEPEDFAVYYCQQHYSSPFTFGQGTKLEIKRTVAAPSVFIFPPSDEQLKSGTASVVCLLNNFYPREAKVQWKVDNALQSGNSQESVTEQDSKDSTYSLSSTLTLSKADYEKHKVYACEVTHQGLSSPVTKSFNRGEC

SEQ ID NO: 49 - protein, 16 aa, Synthetic
AIWGDGSTNYHSALIS